European Patent Specification EP 3 884 023 B1, published July 17, 2024. Title: Detergent Composition. Applicant: Unilever. The sequence listing filed with the application follows.

SEQUENCE LISTING (1 sequence)

SEQ ID NO: 1 - protein, 655 aa, Dictyostelium purpureum
MSLSSSTTNSNSKNKKGNHKSDKVYDLTPYDAPRLQGFLLKSTVFLCESHYLKNSFLSTLYVKNKVPVITQFNTDNMPTFYPIVEKQPEGDFKFKKYFAEDIFLDQNLIDICQSSSQNESSSSSSSSNINIPENNSIFIYNKLYKSNKASPNDILNNFIEVKNHSDEQSPPLAAFIKVLESDIKEQANQSSERWKNKEPLSILDGVPISIKDELDQIGYHTTCGTTFLSKCYPNVKEEDSFVAKKLRERGAILVGKNNMHEIGISTLGYNTHFGFTRNPYNINHYPGGSSSGSAASVSSGLNPISIGCDGGGSIRVPASLCGVVGIKPTFARVSHGGVFELCYSVGHIGPIGSCVVDTAVGYACIAGADPKDPQSVTAEQLGGKPTLPIFTEIPMEQPLKGLKIGIFKDWINDCIEDIKEQTYKCIDILREQGAEIVEIEIPNLLVSRISQLVLILSEMKTSMKRFKNHNNEFQLDSRISLAIAGMFTAEDYIQSNRIRTYCIEELKKIFTNVDAIVTPTNGVVAPEIEKGVPQLGEVNIRAVGDLMKFVFLGNISGIPGISIPIGVTKQNNLPIGFQIMGKWWEEDLLFYISFVLERNIKFNGKPQYFNSPLKVSIENNNSNSNNNNNESTNENNKENNTNIPTNNNEENKSDK